European Patent Application EP 4 316 595 A2, published February 7, 2024. Title: USE OF CGRP RECEPTOR ANTAGONISTS IN NEUROPROTECTION AND NEUROLOGICAL DISORDERS. Applicant: Soares, Christopher J. The sequence listing filed with the application follows.

SEQUENCE LISTING (58 sequences)

SEQ ID NO: 1 - protein, 32 aa, synthetic construct
  REGION 1..32: note = Synthetic peptide
ACDTAACVLGRLSQELHRLQTYPRTNVGSKAF

SEQ ID NO: 2 - protein, 32 aa, synthetic construct
  REGION 1..32: note = Synthetic peptide
ACDTASCVLGRLSQELHRLQTYPRTNVGSKAF

SEQ ID NO: 3 - protein, 32 aa, synthetic construct
  REGION 1..32: note = Synthetic peptide
ACDTAVCVLGRLSQELHRLQTYPRTNVGSKAF

SEQ ID NO: 4 - protein, 32 aa, synthetic construct
  REGION 1..32: note = Synthetic peptide
ACNTAACVLGRLSQELHRLQTYPRTNVGSKAF

SEQ ID NO: 5 - protein, 32 aa, synthetic construct
  REGION 1..32: note = Synthetic peptide
ACVLGACVLGRLSQELHRLQTYPRTNVGSKAF

SEQ ID NO: 6 - protein, 32 aa, synthetic construct
  REGION 1..32: note = Synthetic peptide
ACRFGACVLGRLSQELHRLQTYPRTNVGSKAF

SEQ ID NO: 7 - protein, 32 aa, synthetic construct
  REGION 1..32: note = Synthetic peptide
ACNLSACVLGRLSQELHRLQTYPRTNVGSKAF

SEQ ID NO: 8 - protein, 32 aa, synthetic construct
  REGION 1..32: note = Synthetic peptide
CSNTAACVLGRLSQELHRLQTYPRTNVGSKAF

SEQ ID NO: 9 - protein, 32 aa, synthetic construct
  REGION 1..32: note = Synthetic peptide
ACDTALCVLGRLSQELHRLQTYPRTNVGSKAF

SEQ ID NO: 10 - protein, 32 aa, synthetic construct
  REGION 1..32: note = Synthetic peptide
ACDTAICVLGRLSQELHRLQTYPRTNVGSKAF

SEQ ID NO: 11 - protein, 32 aa, synthetic construct
  REGION 1..32: note = Synthetic peptide
ACNLSVCVLGRLSQELHRLQTYPRTNVGSKAF

SEQ ID NO: 12 - protein, 32 aa, synthetic construct
  REGION 1..32: note = Synthetic peptide
CSNTAVCVLGRLSQELHRLQTYPRTNVGSKAF

SEQ ID NO: 13 - protein, 31 aa, synthetic construct
  REGION 1..31: note = Synthetic peptide
ACNLSACVLGRLSQELHRLQTYPTNTGSGTP

SEQ ID NO: 14 - protein, 32 aa, synthetic construct
  REGION 1..32: note = Synthetic peptide
ACVLGACVLGRLSQELHRLQTYPVDPSSPHSY

SEQ ID NO: 15 - protein, 37 aa, synthetic construct
  REGION 1..37: note = Synthetic peptide
ACDTAACVTHRLAGLLSRSGGVVKNNFVPTNVGSKAF

SEQ ID NO: 16 - skipped

SEQ ID NO: 17 - protein, 7 aa, synthetic construct
  REGION 1..7: note = Synthetic peptide
ACDTAAC

SEQ ID NO: 18 - protein, 7 aa, synthetic construct
  REGION 1..7: note = Synthetic peptide
ACDTASC

SEQ ID NO: 19 - protein, 7 aa, synthetic construct
  REGION 1..7: note = Synthetic peptide
ACDTAVC

SEQ ID NO: 20 - protein, 7 aa, synthetic construct
  REGION 1..7: note = Synthetic peptide
ACNTAAC

SEQ ID NO: 21 - protein, 7 aa, synthetic construct
  REGION 1..7: note = Synthetic peptide
ACVLGAC

SEQ ID NO: 22 - protein, 7 aa, synthetic construct
  REGION 1..7: note = Synthetic peptide
ACRFGAC

SEQ ID NO: 23 - protein, 7 aa, synthetic construct
  REGION 1..7: note = Synthetic peptide
ACDLSAC

SEQ ID NO: 24 - protein, 7 aa, synthetic construct
  REGION 1..7: note = Synthetic peptide
ACNLSAC

SEQ ID NO: 25 - protein, 7 aa, synthetic construct
  REGION 1..7: note = Synthetic peptide
CSNTAAC

SEQ ID NO: 26 - protein, 7 aa, synthetic construct
  REGION 1..7: note = Synthetic peptide
ACDTALC

SEQ ID NO: 27 - protein, 7 aa, synthetic construct
  REGION 1..7: note = Synthetic peptide
ACDTAIC

SEQ ID NO: 28 - protein, 7 aa, synthetic construct
  REGION 1..7: note = Synthetic peptide
ACDTALC

SEQ ID NO: 29 - protein, 7 aa, synthetic construct
  REGION 1..7: note = Synthetic peptide
ACDTAIC

SEQ ID NO: 30 - protein, 7 aa, synthetic construct
  REGION 1..7: note = Synthetic peptide
ACDLSVC

SEQ ID NO: 31 - protein, 7 aa, synthetic construct
  REGION 1..7: note = Synthetic peptide
ACDLSVC

SEQ ID NO: 32 - protein, 7 aa, synthetic construct
  REGION 1..7: note = Synthetic peptide
ACNLSVC

SEQ ID NO: 33 - protein, 7 aa, synthetic construct
  REGION 1..7: note = Synthetic peptide
CSNTAVC

SEQ ID NO: 34 - protein, 19 aa, synthetic construct
  REGION 1..19: note = Synthetic peptide
VLGRLSQELHRLQTYPRTN

SEQ ID NO: 35 - protein, 19 aa, synthetic construct
  REGION 1..19: note = Synthetic peptide
VLGKLSQELHKLQTYPRTN

SEQ ID NO: 36 - protein, 19 aa, synthetic construct
  REGION 1..19: note = Synthetic peptide
VLGKLSQELHKLQTYPRTD

SEQ ID NO: 37 - protein, 19 aa, synthetic construct
  REGION 1..19: note = Synthetic peptide
VLGKLSQELHKLQTFPRTN

SEQ ID NO: 38 - protein, 19 aa, synthetic construct
  REGION 1..19: note = Synthetic peptide
VLGKLSQDIHKLQTYPRTN

SEQ ID NO: 39 - protein, 19 aa, synthetic construct
  REGION 1..19: note = Synthetic peptide
VLGKLSQELHKMQTYPRTD

SEQ ID NO: 40 - protein, 19 aa, synthetic construct
  REGION 1..19: note = Synthetic peptide
LLGKLSQELHRLQTYTRTD

SEQ ID NO: 41 - protein, 19 aa, synthetic construct
  REGION 1..19: note = Synthetic peptide
VLGKLSQDLHKLQTFPRTD

SEQ ID NO: 42 - protein, 19 aa, synthetic construct
  REGION 1..19: note = Synthetic peptide
MLGKLSQDLHKLQTFPRTD

SEQ ID NO: 43 - protein, 19 aa, synthetic construct
  REGION 1..19: note = Synthetic peptide
VLGKLSQDIHKLQTHPRTD

SEQ ID NO: 44 - protein, 19 aa, synthetic construct
  REGION 1..19: note = Synthetic peptide
VLGKLSQDIHKLQTHPRTD

SEQ ID NO: 45 - skipped

SEQ ID NO: 46 - protein, 6 aa, synthetic construct
  REGION 1..6: note = Synthetic peptide
VGSKAF

SEQ ID NO: 47 - protein, 6 aa, synthetic construct
  REGION 1..6: note = Synthetic peptide
VGSKAF

SEQ ID NO: 48 - skipped

SEQ ID NO: 49 - protein, 7 aa, synthetic construct
  REGION 1..7: note = Synthetic peptide
  VARIANT 6: note = Xaa = any amino acid residue other than Thr
ACDTAXC

SEQ ID NO: 50 - protein, 16 aa, synthetic construct
  REGION 1..16: note = Synthetic peptide
EAAAKEAAAKEAAAKA

SEQ ID NO: 51 - protein, 17 aa, synthetic construct
  REGION 1..17: note = Synthetic peptide
AKAAAEKAAAEKAAAEA

SEQ ID NO: 52 - protein, 16 aa, synthetic construct
  REGION 1..16: note = Synthetic peptide
AEAAKAEAAKAEAAKA

SEQ ID NO: 53 - protein, 16 aa, synthetic construct
  REGION 1..16: note = Synthetic peptide
AKAAEAKAAEAKAAEA

SEQ ID NO: 54-56 - skipped (3 entries)

SEQ ID NO: 57 - protein, 32 aa, synthetic construct
  REGION 1..32: note = Synthetic peptide
ACDLSACVLGRLSQELHRLQTYPRTNVGSKAF

SEQ ID NO: 58 - protein, 32 aa, synthetic construct
  REGION 1..32: note = Synthetic peptide
ACDLSVCVLGRLSQELHRLQTYPRTNVGSKAF